European Patent Specification EP 3 765 491 B1, published April 3, 2024. Title: INDUCIBLE T CELL RECEPTORS AND USES THEREOF. Applicant: Medigene Immunotherapies GmbH. The sequence listing filed with the application follows.

SEQUENCE LISTING (12 sequences)

SEQ ID NO: 1 - DNA, 420 bp, Homo sapiens
atccagaatccggaccccgccgtgtaccagctgagagacagcaagagcagcgacaagagtgtgtgcctgttcaccgacttcgactcccagaccaacgtgtcccagagcaaggacagcgacgtgtacatcaccgacaagaccgtgctggacatgcggagcatggacttcaagagcaacagcgccgtggcctggtccaacaagagcgatttcgcctgcgccaacgccttcaacaacagcattatccccgaggacacattcttcccaagccccgagagcagctgcgacgtgaagctggtggaaaagagcttcgagacagacaccaacctgaatttccagaacctgagcgtgatcggcttcagaatcctgctgctgaaggtggccggcttcaacctgctgatgaccctgcggctgtggtccagc

SEQ ID NO: 2 - protein, 140 aa, Homo sapiens
IQNPDPAVYQLRDSKSSDKSVCLFTDFDSQTNVSQSKDSDVYITDKTVLDMRSMDFKSNSAVAWSNKSDFACANAFNNSIIPEDTFFPSPESSCDVKLVEKSFETDTNLNFQNLSVIGFRILLLKVAGFNLLMTLRLWSS

SEQ ID NO: 3 - DNA, 537 bp, Homo sapiens
gaagatctgaagaacgtgttccccccagaggtggccgtgttcgagcctagcgaggccgagatcagccacacccagaaagccaccctcgtgtgcctggccaccggcttctatcccgaccacgtggaactgtcttggtgggtcaacggcaaagaggtgcacagcggcgtgtccaccgatccccagcctctgaaagaacagcccgccctgaacgacagccggtactgcctgagcagccggctgagagtgtccgccaccttctggcagaacccccggaaccacttcagatgccaggtgcagttctacggcctgagcgagaacgacgagtggacccaggacagagccaagcccgtgacccagatcgtgtctgccgaagcctggggcagagccgattgcggctttaccagcgagagctaccagcagggcgtgctgagcgccaccatcctgtacgagatcctgctgggcaaggccaccctgtacgccgtgctggtgtctgccctggtgctgatggctatggtcaagcggaaggacagccggggc

SEQ ID NO: 4 - protein, 179 aa, Homo sapiens
EDLKNVFPPEVAVFEPSEAEISHTQKATLVCLATGFYPDHVELSWWVNGKEVHSGVSTDPQPLKEQPALNDSRYCLSSRLRVSATFWQNPRNHFRCQVQFYGLSENDEWTQDRAKPVTQIVSAEAWGRADCGFTSESYQQGVLSATILYEILLGKATLYAVLVSALVLMAMVKRKDSRG

SEQ ID NO: 5 - protein, 140 aa, Artificial Sequence
  Amino acid sequence of nucleic acid sequence A
IQNPDPAVYQLRDSKSSDKSVCLFTDFDSQTNVSQSKDSDVYIADKAVLDMRSMDFKSNSAVAWSNKSDFACANAFNNSIIPEDTFFPSPESSCDVKLVEKSFETDTNLNFQNLSVIGFRILLLKVAGFNLLMTLRLWSS

SEQ ID NO: 6 - protein, 179 aa, Artificial Sequence
  Amino acid sequence of nucleic acid sequence B
EDLKNVFPPEVAVFEPSEAEISHTQKATLVCLATGFYPDHVELSWWVNGKEVHSGVSTDPQPAKEQPALNDSRYCLASALRVSATFWQNPRNHFRCQVQFYGLSENDEWTQDRAKPVTQIVSAEAWGRADCGFTSESYQQGVLSATILYEILLGKATLYAVLVSALVLMAMVKRKDSRG

SEQ ID NO: 7 - DNA, 930 bp, Artificial Sequence
  ERT2
atgagagccgccaatctgtggcccagccccctgatgatcaagcggagcaagaagaactccctggccctgagcctgaccgccgaccagatggtgtcagctctgctggatgccgagccccctatcctgtacagcgagtacgaccccacccggccttttagcgaggccagcatgatgggcctgctgaccaatctggccgaccgcgagctggtgcacatgatcaactgggccaagcgggtgcccggcttcgtggatctgacactgcacgaccaggtgcacctgctggaatgcgcctggctggaaatcctgatgattggcctcgtgtggcggagcatggaacaccccgtgaagctgctgttcgcccccaacctgctgctggaccggaaccagggcaaatgcgtggaaggcatggtggaaatcttcgacatgctgctggccacctccagccggttcagaatgatgaacctgcagggcgaagagttcgtgtgtctgaagtccatcatcctgctgaacagcggcgtgtacaccttcctgagcagcaccctgaagtccctggaagagaaggaccacatccaccgggtgctggacaagatcaccgacaccctgatccacctgatggctaaggccggactgaccctgcagcagcagcatcagagactggcccagctgctgctgatcctgagccacatccggcacatgagcaacaagggaatggaacatctgtacagcatgaagtgcaagaacgtggtgcccctgtacgatctgctgctggaagccgccgatgcccacagactgcacgcccctacatctagaggcggagccagcgtggaagagacagaccagtctcacctggccacagccggctccacaagctctcacagcctgcagaagtactacatcaccggcgaggccgagggctttcctgcaacagcc

SEQ ID NO: 8 - protein, 310 aa, Artificial Sequence
  ERT2
MRAANLWPSPLMIKRSKKNSLALSLTADQMVSALLDAEPPILYSEYDPTRPFSEASMMGLLTNLADRELVHMINWAKRVPGFVDLTLHDQVHLLECAWLEILMIGLVWRSMEHPVKLLFAPNLLLDRNQGKCVEGMVEIFDMLLATSSRFRMMNLQGEEFVCLKSIILLNSGVYTFLSSTLKSLEEKDHIHRVLDKITDTLIHLMAKAGLTLQQQHQRLAQLLLILSHIRHMSNKGMEHLYSMKCKNVVPLYDLLLEAADAHRLHAPTSRGGASVEETDQSHLATAGSTSSHSLQKYYITGEAEGFPATA

SEQ ID NO: 9 - protein, 15 aa, Artificial Sequence
  relevant "TDA" peptide
TDAWRFAMNYPRNPT

SEQ ID NO: 10 - protein, 13 aa, Artificial Sequence
  irrelevant "PEV" peptide
PEVWILSPLLRHG

SEQ ID NO: 11 - protein, 9 aa, Artificial Sequence
  irrelevant T2 peptide
VLDGLDVLL

SEQ ID NO: 12 - protein, 9 aa, Artificial Sequence
  relevant T2 peptide
SLLMWITQC